European Patent Specification EP 4 103 611 B1, published March 27, 2024. Title: Antibodies. Applicant: UCB Biopharma SRL. The sequence listing filed with the application follows.

SEQUENCE LISTING (22 sequences)

SEQ ID NO: 1 - protein, 283 aa, homo sapiens
MEPPGDWGPPPWRSTPKTDVLRLVLYLTFLGAPCYAPALPSCKEDEYPVGSECCPKCSPGYRVKEACGELTGTVCEPCPPGTYIAHLNGLSKCLQCQMCDPAMGLRASRNCSRTENAVCGCSPGHFCIVQDGDHCAACRAYATSSPGQRVQKGGTESQDTLCQNCPPGTFSPNGTLEECQHQTKCSWLVTKAGAGTSSSHWVWWFLSGSLVIVIVCSTVGLIICVKRRKPRGDVVKVIVSVQRKRQEAEGEATVIEALQAPPDVTTVAVEETIPSFTGRSPNH

SEQ ID NO: 2 - protein, 228 aa, Homo sapiens
MPVKGGTKCIKYLLFGFNFIFWLAGIAVLAIGLWLRFDSQTKSIFEQETNNNNSSFYTGVYILIGAGALMMLVGFLGCCGAVQESQCMLGLFFGFLLVIFAIEIAAAIWGYSHKDEVIKEVQEFYKDTYNKLKTKDEPQRETLKAIHYALNCCGLAGGVEQFISDICPKKDVLETFTVKSCPDAIKEVFDNKFHIIGAVGIGIAVVMIFGMIFSMILCCAIRRNREMV

SEQ ID NO: 3 - protein, 10 aa, Artificial Sequence
  CDR-H1 VR7660
GFSLSTYDMI

SEQ ID NO: 4 - protein, 16 aa, Artificial Sequence
  CDR-H2 VR7660
VITKTTTTYYANWAKG

SEQ ID NO: 5 - protein, 12 aa, Artificial Sequence
  CDR-H3 VR7660
DADDAVYYYFDI

SEQ ID NO: 6 - protein, 11 aa, Artificial Sequence
  CDR-L1
QASQSIGSGLA

SEQ ID NO: 7 - protein, 7 aa, Artificial Sequence
  CDR-L2 VR7660
AASTLTS

SEQ ID NO: 8 - protein, 12 aa, Artificial Sequence
  CDR-L3 VR7660
QEGVSRGNIDNA

SEQ ID NO: 9 - protein, 10 aa, Artificial Sequence
  CDR-H1 VR7272
GFSLSSYAMG

SEQ ID NO: 10 - protein, 16 aa, Artificial Sequence
  CDR-H2 VR7272
AIGSITATGYARWAKG

SEQ ID NO: 11 - protein, 12 aa, Artificial Sequence
  CDR-H3 VR7272
EIYVGSAYAFDI

SEQ ID NO: 12 - protein, 11 aa, Artificial Sequence
  CDR-L1 VR7272
QASQSISNYLA

SEQ ID NO: 13 - protein, 7 aa, Artificial Sequence
  CDR-L2 VR7272
LASTLAS

SEQ ID NO: 14 - protein, 11 aa, Artificial Sequence
  CDR-L3 VR7272
QQGYIDNVNKG

SEQ ID NO: 15 - protein, 117 aa, Artificial Sequence
  VH VR7660
QSVEESGGRLVTPGTPLTLTCTVAGFSLSTYDMIWVRQAPGKGLEYIGVITKTTTTYYANWAKGRFTISKTSTTVDLKMTSPTTEDTATYFCARDADDAVYYYFDIWGPGTLVTVSS

SEQ ID NO: 16 - DNA, 424 bp, Artificial Sequence
  VH nucl VR7660
aagcttcgaagccaccatggagactgggctgcgctggcttctcctggtcgctgtgctcaaaggtgtccagtgtcagtcggtggaggagtccgggggtcgcctggtcacgcctgggacacccctgacactcacctgcacggtcgctggattctccctcagtacctacgacatgatctgggtccgccaggctccagggaaggggctggaatacatcggagtcattactaaaactactaccacatactacgcgaactgggcgaaaggccgattcaccatctccaaaacctcgaccacggtggatctgaaaatgaccagtccgacaaccgaggacacggccacctatttctgtgccagagatgctgatgatgctgtttattactactttgacatctggggcccaggcaccctggtcaccgtctcgagt

SEQ ID NO: 17 - protein, 110 aa, Artificial Sequence
  VL VR7660
AYDMTQTPASAEVAVGGTVTINCQASQSIGSGLAWYQQKPGQRPKLLIYAASTLTSGVSSRFKGSGSGTEFTLTISGVECADAATYYCQEGVSRGNIDNAFGGGTEVVVK

SEQ ID NO: 18 - DNA, 418 bp, Artificial Sequence
  VL nucl VR7660
aagcttcgaagccaccatggacatgagggcccccactcagctgctggggctcctgctgctctggctcccaggtgccagatgtgcctatgatatgacccagactccagcctctgcggaggtagctgtgggaggcacagtcaccatcaattgccaggccagtcagagcattggcagtggtttggcctggtatcagcagaaaccagggcagcgtcccaaactcctgatctatgctgcatccactctgacatctggggtctcatcgcggttcaaaggcagtggatctgggacagagttcactctcaccatcagcggcgtggagtgtgccgatgctgccacttactactgtcaagagggtgttagtcgtggtaatattgataatgccttcggcggagggaccgaggtggtggtcaaacgtacg

SEQ ID NO: 19 - protein, 117 aa, Artificial Sequence
  VH VR7272
QSLEESGGRLVTPGTPLTLTCTVSGFSLSSYAMGWVRQAPGKGLEWIGAIGSITATGYARWAKGRFSISKTSTTVDLKMTSPTTEDTATYFCAREIYVGSAYAFDIWGPGTLVTVSS

SEQ ID NO: 20 - DNA, 424 bp, Artificial Sequence
  VH nucl VR7272
aagcttcgaagccaccatggagactgggctgcgctggcttctcctggtcgctgtgctcaaaggtgtccagtgtcagtcgctggaggagtccgggggtcgcctggtcacgcctgggacacccctgacactcacctgcacagtctctggattctccctcagtagctatgcaatgggctgggtccgccaggctccagggaaggggctggagtggatcggagccattggtagtattactgccactggctacgcgcgctgggcaaaaggccgattcagcatctccaagacctcgaccacggtggatctgaaaatgaccagtccgacaaccgaggacacggccacctatttctgtgccagagagatttatgttgggtctgcttatgcctttgacatctggggcccaggcaccctggtcaccgtctcgagt

SEQ ID NO: 21 - protein, 109 aa, Artificial Sequence
  VL VR7272
AYDMTQTPASVEVAVGDTVTIKCQASQSISNYLAWYQQKPGQPPKLLIYLASTLASGVPSRFKGSGSGTEFTLTISDLECADAATYYCQQGYIDNVNKGFGGGTEVVVK

SEQ ID NO: 22 - DNA, 415 bp, Artificial Sequence
  VL nucl VR7272
aagcttcgaagccaccatggacacgagggcccccactcagctgctggggctcctgctgctctggctcccaggtgccagatgtgcctatgatatgacccagactccagcctctgtggaggtagctgtgggagacactgtcaccatcaagtgtcaggccagtcagagcattagtaactacttagcctggtatcagcagaaaccagggcagcctcccaagctcctgatctatctggcatctactctggcatctggggtcccatcgcggttcaaaggcagtggatctgggacagagttcactctcaccatcagcgacctggagtgtgccgatgctgccacttactattgtcaacagggttatattgataatgttaataaaggtttcggcggagggaccgaggtggtggtcaaacgtacg